European Patent Specification EP 3 744 725 B1, published September 17, 2025. Title: Diversification of Human Milk Oligosaccharides (HMOs) or Precursors Thereof. Applicant: Glycom A/S. The sequence listing filed with the application follows.

SEQUENCE LISTING (21 sequences)

SEQ ID NO: 1 - protein, 448 aa, Thermotoga maritima
  SOURCE 1..448: /mol_type="protein" /note="gi|4980806|gb|AAD35394.1|AE001712_7 alpha-L-fucosidase, pu tative " /organism="Thermotoga maritima"
MISMKPRYKPDWESLREHTVPKWFDKAKFGIFIHWGIYSVPGWATPTGELGKVPMDAWFFQNPYAEWYENSLRIKESPTWEYHVKTYGENFEYEKFADLFTAEKWDPQEWADLFKKAGAKYVIPTTKHHDGFCLWGTKYTDFNSVKRGPKRDLVGDLAKAVREAGLRFGVYYSGGLDWRFTTEPIRYPEDLSYIRPNTYEYADYAYKQVMELVDLYLPDVLWNDMGWPEKGKEDLKYLFAYYYNKHPEGSVNDRWGVPHWDFKTAEYHVNYPGDLPGYKWEFTRGIGLSFGYNRNEGPEHMLSVEQLVYTLVDVVSKGGNLLLNVGPKGDGTIPDLQKERLLGLGEWLRKYGDAIYGTSVWERCCAKTEDGTEIRFTRKCNRIFVIFLGIPTGEKIVIEDLNLSAGTVRHFLTGERLSFKNVGKNLEITVPKKLLETDSITLVLEAVE

SEQ ID NO: 2 - protein, 403 aa, Sulfolobus solfataricus
  SOURCE 1..403: /mol_type="protein" /note=">gi|13816464|gb|AAK43159.1| Alpha-fucosidase C-terminal fr agment (fucA1)" /organism="Sulfolobus solfataricus"
MFTGENWDPYEWAKVFKKSGAKFVVLVAEHHDGFALWESNYTRWCATKIGPKRDIVRELKEAVEGQGLIFGISYHRAEHWWFFDQGMKIESDVKDPRYLDLYGPAQSASLNPRDPPSLDNVQPNDEFLMDWLLRIVEAVEKYRPWLVYFDWWIANPSFQPYLKAFASYYYNRSYKWGIEPVIIYKQGAFGEGTAIPDLAERGTIKNVYPSTWLADTSIDYKSWGYIKDAEYKLPSVILSHLGDVVSKNGVFLLNIGPKADGTIPEEAKRILLDVGDWLNVNGEAIFGSKPWRVYGEGPSGINEGGFFTERKITLGYQDVRYTVKDYYPRQRHIYAILFGKPKEITLRSFMKNLKLIEEAVIVDVSRLDGKGKLEWSLSDEGLKIKIEEVIRAPLVIRVILDYR

SEQ ID NO: 3 - protein, 1959 aa, Bifidobacterium bifidum
  SOURCE 1..1959: /mol_type="protein" /note=">gi|34451973|gb|AAQ72464.1| alpha-fucosidase " /organism="Bifidobacterium bifidum"
MKHRAMSSRLMPLVASCATVGMLLAGLPVSAVAVGTTRAAASDASSSTTATITPSADTTLQTWTSEKNSSMASKPYIGTLQGPSQGVFGEKFESTDAADTTDLKTGLLTFDLSAYDHAPDSATFEMTYLGYRGNPTATDTDTIKVTPVDTTVCTNNATDCGANVATGATKPKFSINDSSFVAESKPFEYGTTVYTGDAITVVPANTKKVTVDVTEIVRQQFAEGKKVITLAVGETKKTEVRFASSEGTTSLNGATADMAPKLTVSVSTKDDLKPSADTTLQAWASEKNEKKNTAAYVGALQPEGDYGDFGEKFKSTDVHDVTDAKMGLMTFDLSDYTAAPEHSILTLTYLGYAGADKTATATDKVKVVAVDTSRCTGTAPCDTNNATWANRPDFEVTDTTKTATSHAFAYGSKKYSDGMTVESGNAKKVLLDVSDVIKAEFAKFSAGATEKKITLALGELNKSDMRFGSKEVTSLTGATEAMQPTLSVTKKPKAYTLSIEGPTKVKYQKGEAFDKAGLVVKATSTADGTVKTLTEGNGEDNYTIDTSAFDSASIGVYPVTVKYNKDPEIAASFNAYVIASVEDGGDGDTSKDDWLWYKQPASQTDATATAGGNYGNPDNNRWQQTTLPFGNGKIGGTVWGEVSRERVTFNEETLWTGGPGSSTSYNGGNNETKGQNGATLRALNKQLANGAETVNPGNLTGGENAAEQGNYLNWGDIYLDYGFNDTTVTEYRRDLNLSKGKADVTFKHDGVTYTREYFASNPDNVMVARLTASKAGKLNFNVSMPTNTNYSKTGETTTVKGDTLTVKGALGNNGLLYNSQIKVVLDNGEGTLSEGSDGASLKVSDAKAVTLYIAAATDYKQKYPSYRTGETAAEVNTRVAKVVQDAANKGYTAVKKAHIDDHSAIYDRVKIDLGQSGHSSDGAVATDALLKAYQRGSATTAQKRELETLVYKYGRYLTIGSSRENSQLPSNLQGIWSVTAGDNAHGNTPWGSDFHMNVNLQMNYWPTYSANMGELAEPLIEYVEGLVKPGRVTAKVYAGAETTNPETTPIGEGEGYMAHTENTAYGWTAPGQSFSWGWSPAAVPWILQNVYEAYEYSGDPALLDRVYALLKEESHFYVNYMLHKAGSSSGDRLTTGVAYSPEQGPLGTDGNTYESSLVWQMLNDAIEAAKAKGDPDGLVGNTTDCSADNWAKNDSGNFTDANANRSWSCAKSLLKPIEVGDSGQIKEWYFEGALGKKKDGSTISGYQADNQHRHMSHLLGLFPGDLITIDNSEYMDAAKTSLRYRCFKGNVLQSNTGWAIGQRINSWARTGDGNTTYQLVELQLKNAMYANLFDYHAPFQIDGNFGNTSGVDEMLLQSNSTFTDTAGKKYVNYTNILPALPDAWAGGSVSGLVARGNFTVGTTWKNGKATEVRLTSNKGKQAAVKITAGGAQNYEVKNGDTAVNAKVVTNADGASLLVFDTTAGTTYTITKKASANVPVTGVTVTGANTATAGDTVTLTATVAPANATDKSVTWSTSDAAVATVNANGVVTTKKAGKVTITATSNGDKTKFGSIEITVSAATVPVTSVTVAGDAAMTVDGEQTLTATVAPATATDKTVTWKSSDATVATVDANGKVVAKKAGEVTITATAGGVSGTLKITVSDKAPTVIPVQSVTVTGKQELVEGASTTLTATVAPADATDKTVTWKSSDESVATVDKDGVVTAKKAGTVTITATAGGVSGTLHITVTAKPVETVPVTSVEVTVEAGTTVSVGKTLQATATVKPGNATNKKVTWKSSDESIATVDANGVITAKKAGKVVITATSTDGTDKSGSVEITVVDETKPTPDHKSVKADTGDVTAGKTGTVTEPKDVAGWKSRSIIKQGKLGKAEIADGTLVYAAGDKTGDDSFVVQYTMADGTVIDVTYSVTVKAAETGKNDGDGKGDGVAKTGAAVGALAGLGLMLLAVGVSVVMIRRKHSA

SEQ ID NO: 4 - protein, 1493 aa, Bifidobacterium bifidum
  SOURCE 1..1493: /mol_type="protein" /note="gi|242345155|dbj|BAH80310.1| alpha-L-fucosidase [Bifidobac terium bifidum JCM 1254]" /organism="Bifidobacterium bifidum"
MLHTASRGCSRSWLRRLTALIAVSALAFVALPNVAVAADPMEYLDVSFGGTFAADTYTTGGDEVAKGPVTKHGSIPTKLDGGGITLAGGTNGVTFTSTASFSESGKVNKGFRAEMEYRTTQTPSNLATLFSAMGNIFVRANGSNLEYGFSTNPSGSTWNDYTKSVTLPSNNVKHIIQLTYLPGADGAASTLQLSVDGVAGETATSAAGELAAVSDSVGNKFGIGYEVNPASGAASRGLAGDVFRARVADSDAPWEILDASQLLHVNFNGTFSGTSYTAASGEQMLGSLVSRSANPSISNSAVTLGGGTAGFDFTPTDFTLGDNEAITRPLVAELRFTPTQTGDNQTLFGAGGNLFLRYESNKLVFGASTKSGDNWTDHKIESAAATGAEHVVSVAYVPNKAGTGAKLVMRVDGGDAQTKDITGLAYLNSSIKGKVGFGNDVHTDALSRGFVGSLSEIRLAETSANFTTNEFKLVYSQVSCDTSGIKEANTFDVEPAECEAALKTKLSKLRPTEGQADYIDWGQIGFLHYGINTYYNQEWGHGNEDPSRINPTGLDTDQWAKSFADGGFKMIMVTVKHHDGFELYDSRYNTEHDWANTAVAKRTGEKDLFRKIVASAKKYGLKVGIYYSPADSYMERKGVWGNNSARVERTIPTLVENDDRAGKVASGKLPTFKYKATDYGAYMLNQLYELLTEYGDISEVWFDGAQGNTAGTEHYDYGVFYEMIRRLQPQAIQANAAYDARWVGNEDGWARQTEWSPQAAYNDGVDKVSLKPGQMAPDGKLGSMSSVLSEIRSGAANQLHWYPAEVDAKNRPGWFYRASQSPASVAEVVKYYEQSTGRNSQYLLNVPPSDTGKLADADAAGLKGLGEELARRYGTDLALGKSATVAASANDTAVAAPKLTDGSKLSSDKAVGNTPTYTIDLGSTVAVDAVKISEDVRNAGQQIESATLQGRVNGTWTNLATMTTVGQQRDLRFTSQNIDAIRLVVNSSRGPVRLSRLEVFHTESEIQTGARAYYIDPTAQTAGDGFTKDKPMTSIEQLHDVTVAPGSVIFVKAGTELTGDFAVFGYGTKDEPITVTTYGESDKATTASFDGMTAGLTLKQALKALGKDDAGWVVADSATAPASRVYVPQDEISVHAQSSQNSGAEAARALDGDSSTSWHSQYSPTTASAPHWVTLDLGKSRENVAYFDYLARIDGNNNGAAKDYEVYVSDDPNDFGAPVASGTLKNVAYTQRIKLTPKNGRYVKFVIKTDYSGSNFGSAAEMNVELLPTAVEEDKVATPQKPTVDDDADTYTIPDIEGVVYKVDGKVLAAGSVVNVGDEDVTVTVTAEPADGYRFPDGVTSPVTYELTFTKKGGEKPPTEVNKDKLHATITKAQAIDRSAYTDESLKVLDDKLAAALKVYDDDKVSQDDVDAAEAALSAAIDALKTKPTTPGGEGEKPGEGEKPGDGNKPGDGKKPGDVIAKTGASTMGVVFAALAMVAGAVVTLEAKRKSNR

SEQ ID NO: 5 - protein, 478 aa, Bifidobacterium longum subsp. infantis
  SOURCE 1..478: /mol_type="protein" /note="gi|213524647|gb|ACJ53394.1| alpha-1,3/4-fucosidase, putati ve [Bifidobacterium longum subsp. infantis ATCC 15697]" /organism="Bifidobacterium longum subsp. infantis"
MNNPADAGINLNYLANVRPSSRQLAWQRMEMYAFLHFGMNTMTDREWGLGHEDPALFNPRNVDVDQWMDALVAGGMAGVILTCKHHDGFCLWPSRLTRHTVASSPWREGKGDLVREVSESARRHGLKFGVYLSPWDRTEESYGKGKAYDDFYVGQLTELLTQYGPIFSVWLDGANGEGKNGKTQYYDWDRYYNVIRSLQPDAVISVCGPDVRWAGNEAGHVRDNEWSVVPRRLRSAELTMEKSQQEDDASFATTVSSQDDDLGSREAVAGYGDNVCWYPAEVDTSIRPGWFYHQSEDDKVMSADQLFDLWLSAVGGNSSLLLNIPPSPEGLLAEPDVQSLKGLGRRVSEFREALASVRCEARTSSASAAAAHLVDGNRDTFWRPDADDAAPAITLTLPQPTTINAIVIEEAIEHGQRIEHLRVTGALPDGTERVLGQAGTVGYRRILRFDDVEVSSVTLHVDGSRLAPMISRAAAVRI

SEQ ID NO: 6 - protein, 378 aa, Lactobacillus casei
  SOURCE 1..378: /mol_type="protein" /note="gi|190713109|emb|CAQ67115.1| Alpha-L-fucosidase [Lactobaci llus casei BL23]" /organism="Lactobacillus casei"
MTKPSAVNIHRTNPPDWFKQADFGIIIHWGPYSVPAYAPVNIPDYGTLIKTKSLGYLFEHQPYAEWYGNSMLLPSSPVAAYHRTHYGNTSYADFAKTFKQTAQNVDVQAWAAAFANAGAKYVVIVTKHHDGFVMFDPHTKNPYEPDYHLNFDFVGELAQAVRAHGMRFGTYYSSLLDWTFPHLPIKDYGSFLLGNDKSQTYKDYVWHQWHELIDRYHPDVLWNDIGYPDDHRLETLFKYYYQQVPEGLVNDRWQQFPDWMRTSWIRPIFNLVAAQVIKRDQHHSNDLSEVKYYDYRTFEYRTDWPQTNRYFEMTRGMDKSFGYNRLSRPEDYITADDIKQLIAELRSKRGRLLLNVGPDMNGQIPSAQLSILQQLSDR

SEQ ID NO: 7 - protein, 414 aa, Lactobacillus casei
  SOURCE 1..414: /mol_type="protein" /note="gi|190713871|emb|CAQ67877.1| Alpha-L-fucosidase [Lactobaci llus casei BL23]" /organism="Lactobacillus casei"
MTEPLPRIQHYEDLGLGLFIHWGLYSQMAVGEWTELIHHRNQHDYEQLIKTFTAAQFDAKKIAHAAKAVGAKYIVLTTKHHEGFFLYDTKGLSDFDVMHAPARRDLIAEFVAACREEDLLPFFYMATYDWHTPLYDDDFPAYLTYLQKSVEVLCRNYGPVGGFWFDGNWNKKDADWHLPELYGMIRHYQPNAIIVNNTGLKNRGQVSDPEIDVVTYERRTPDEIYHGAPNEKYVAGEISITLNQHWGIAANDLNYKSPAEVIETVAHARHIGANILVNIGLTGTGAIPAAAQTYMHLLGRWTAMAAPVLYKGRPVPVTSAHGTRDFVLHTSKHDFLCILDLQVVGNDNVVLGGEGVNPRSFVGIGQPIQRIHWLDNDEVLSFTQDLDKKVLTVDATGYPYGSDWVVRIAQIDYE

SEQ ID NO: 8 - protein, 344 aa, Lactobacillus casei
  SOURCE 1..344: /mol_type="protein" /note="gi|190713978|emb|CAQ67984.1| Alpha-L-fucosidase [Lactobaci llus casei BL23]" /organism="Lactobacillus casei"
MNDNVAWFKQAKYGMMIHWGLYSLLAGEYRGESSSAYAEWIQSKFQIPNAEYGNLATAFNPLYFDAKKIVALAKQCGMQYLVVTTKHHDGFAMYHSKVDAYNVYDATPFHRDIIGELAEACQKAGLKFGLYYSQDLDWHDPNGGGYKSNDVETAGTTWDNSWDFPDEDQKNFDLCFDNKILPQIKEIMSNYGDIATAWFDVPMTLSEAQSQTIYDTVRELQPNCLINSRLGNGKYDFVSLGDNEIPKNKEDMNKTDVDYNEITGFKPSPLGLYETAGTINDSWGFSYHDQNWKTPRTLYRYKQHLNDFGINYLLNVGLDPLGRVPMMAEENLLAAKALEDEANR

SEQ ID NO: 9 - protein, 1795 aa, Bifidobacterium bifidum
  SOURCE 1..1795: /mol_type="protein" /note="gi|310867437|gb|ADP36806.1| Exo-alpha-sialidase [Bifidobac terium bifidum PRL2010]" /organism="Bifidobacterium bifidum"
MTTIFRRATAKTLMRKLSGLLVAIAMLAVLPAGTISANAADEPPQEYLQLTLTRTDSNGTPAEVGDKLTYSLGYKNVSDTGFIVHPTASNLNNVATPQSASNPNPMCRWGNLAAGASAACTWSASKEFAYHVVTEDDVANGFTPTATVSATTQDGTNGVLQSVDITGETVPAVPATSTLRVAMQRTDTLGDNVKIGDRLTFNFTYTNKTAQKIYAYPSESNIERVDVVSFPRNSCRSGVEANQTASCGFAYHVITAEDVVARRYTPTATFRATSDRDGTQVLQDDMTFTTGTVTVAGPADDAASTPTERKDGEPLLLATNKQIGNTDYYRIPAIAQAPNGWILAAWDLRPKLAADAPNPNSIVQRISKDGGKSWETLAYVAQGRSATNKYGYSDPSYVVDEEAGKIFLFCVKSYDQGYFGSVLGVEDARNVLQAVVMESDDNGATWSEPRNITKDITKGHEDEWKSRFASSGHGIQLKYGQYKGRLIQQYAVRTTSNTNIAVSVYSDDHGKTWKAGNPVTEANMDENKVVELSDGRVMLNSRPGAAGYRRVAISEDGGVNYGPIKSETQLPDPNNNAQITRAFPNAPEGSAKAKVLLYSAPRASNEGRANGVVRVSFDDGTTWSAGKLFKEGSMAYSVITALNDAAGGGYGLLYEGESITYTRVSMEWLGYLTATASGTATVKEGEGTLTAPVTVTNDGLTDYTNVTVTPTGLPSGWSAEAVNVGNLAAGQSATVNVPVTVPAAAVSGTVAKATMKITGKYAQSEDTLHSFAEGELAVTVTEPDPAAKRLKLTIERTDDNGAPVKVGDTLTYRITYENVGTQSFAVYPRKSNLDGVTTPQSASNPAPVCRWSRLDPGTTGACVSGNGKRLAYHTVTEADATAGSFTPSATIDATADTSGETVLESVSITGDPVTVSQPVELPADIAAWKTRNEALDDWQTLSEKLAKTDRINWLFTGDSITHGVQLTRGYRTYSELFANHLDTASVRGVSRANDVVMNTGISSADASWPLKDGAFEKWVSDKHPDVVFLTFGMNDGRTGQAFTVDQYTANLSTLIDKIRDLGAIPVLQTQNYTTNTTFNANLDTYFDAERRLALDKNVLLVDFNKQWLELGGGNRESGTYMGAGNDIHPGENGHIEWAKFTLGALNMIANDDPLARWSSSDTTLDKPTVTVDADGNGLKGSDGLEPAPAAAKSVGKFLSGAQYVDLGGDVVSAVAGKRESNVTIRFRASATGQPQTLFSLGDSDSATRATVRLSATGLVQFLNSGNTGDFYTVGTNDLADGAWHTVSVNFVANGFTIYVDGAAMRAISGGAGTQLNVPGAITVNTATAGAIRGADSAGGAQQLTGIVDYVAAWSRTLTDAEAKRISAETSAVAVTKVDAAVNALQPIISDTGARKNIVFVGGETIEGGYTDHLIAKNIVQLLDERVRWEYVTGLSATDRELQRAKFFVAAGQGGLTAKQMDEDYAAMVGEYSPDILFLAPDLYDADGILAESDAAAFAGHIRSVAAKAKEAGAKVVLVTPVTVRGGEDEYAGAMRTVAKEDDLPLIDAQAWIGKVVAADASVKTAWFNKAGQLNYAGHLGYARFMMRSLDLYPSNVSGSRIASLPYDTANVTLVGASENGGELPVGRVEGTDRAHIDTMQIGAAASLVVTDSYAVYEIGEDGGRTLVADGLKPADVLADGIDVTVNDTAAHRYEVVGSANVPEGADAVTVTYTATLAAVEEPEPGPDPDPTPDPSEKPDGDGTGDGTGAGAGDVQKPTPDAVAKTGADVFGLLAAVAVLLAAGGVTLSLRRRANR

SEQ ID NO: 10 - protein, 770 aa, Bifidobacterium bifidum
  SOURCE 1..770: /mol_type="protein" /note="gi|310867438|gb|ADP36807.1| Exo-alpha-sialidase [Bifidobac terium bifidum PRL2010]" /organism="Bifidobacterium bifidum"
MVRSTKPSLLRRFGALVAAAAMLVVLPAGVSTASAASDDADMLTVTMTRTDALGDEVYVGDTLTYSFTNTNNTSSAFTAFPAESNLSGVLTTGTPNCRYENLAGGASYPCSTASHTITADDLTAGSFTPRTVWKATSDRGGTQVLQDNIVSTGDTVTVKEGKRPDPATIPTDRADGEAVRLATARQNLGTECYRIPALAEAPNGWILAAFDQRPNTAMANGSGVKCWDAPQPNSIVQRISKDGGKSWTPIQYVAQGKNAPERYGYSDPSYVVDKETGEIFLFFVHSYNKGFADSQLGVDESNRNVLHAVVVSSKDNGETWSKPRDITADITKGYENEWKSRFATSGAGIQLKYGKYKGRLIQQYAVGRTTGSNAAVSVYSDDHGKTWQAGNPVTGMLMDENKVVELSDGRVMLNSRPGNGSGYRRVAISEDGGVNYGTVKNETQLPDPNNNAHITRAFPNAPEGSAKAKVLLYSSPRANNEGRANGVVRISLDDGTTWSSGKLYKEGSMAYSVITALSGAAGGGYGLLYEGAWVTGGGIDSHDIMYTHISMDWLGYLSATADDVTASVEEGASTVDVTVPVSNVGSVDYTGVTVTPADLPTGWSASPVNVGALASGASKDVTVTVNVPATAKKDDVAKIVLRVTGTSAANANATTGFDGSITVNVTEKSEPDPEPEPTITGVSAVTSQAGVKVGDVFDASKVSVTAAMSDGSSKALAAGEYSLSAVDADGKAVDLAEPFAAAGVVTVTVSVPVEGADPLTASFTIDVAEK

SEQ ID NO: 11 - protein, 836 aa, Bifidobacterium bifidum
  SOURCE 1..836: /mol_type="protein" /note="gi|309252191|gb|ADO53939.1| sialidase [Bifidobacterium bif idum S17]" /organism="Bifidobacterium bifidum"
MVRSTKPSLLRRLGALVAAAAMLVVLPAGVSTASAASDDADMLTVTMTRTDTLGDEVYVGDTLTYSFTNTNNTSSAFTAFPAESNLSGVLTTGTPNCRYENLAGGASYPCSTASHTITADDLTAGSFTPRTVWKATSDRGGTQVLQDNIVSTGDTVTVKEGKRPDPATIPTDRADGEAVRLATARQNLGTECYRIPALAEAPNGWILAAFDQRPNTAMANGSGVKCWDAPQPNSIVQRISKDGGKSWTPIQYVAQGKNAPERYGYSDPSYVVDEETGEIFLFFVHSYNKGFADSQLGVDESNRNVLHAVVVSSKDNGETWSKPRDITADITKGYENEWKSRFATSGAGIQLKYGKYKGRLIQQYAVGRTTGSNAAVSVYSDDHGKTWQAGNPVTGMLMDENKVVELSDGHVMLNSRPGNGSGYRRVAISEDGGVNYGTVKNETQLPDPNNNAHITRAFPNAPEGSAKAKVLLYSSPRANNEGRANGVVRISLDDGTTWSSGKLYKAGSMAYSVITALSGAAGGGYGLLYEGAWVTGGGIDSHDIMYTHISMDWLGYLSATADDVTASVEEGASTVDVTVPVSNVGSVDYTGVTVTPADLPTGWSASPVNVGALASGASKDVTVTVNVPATAKKDDVAKIVLRVTGTSAANADATTGFDGSITVNVTEKSEPDPEPEPTITGVSAVTSQAGVKVGDVFDASKVSVTAAMSDGSSKALAAGEYSLSAVDADGKAVDLAEPFAAAGVVTVTVSVPVEGADPLTASFTIDVAEKSADPEPKPEPEPKPEPEKPAGPKVDVPTEKPGLSKTGASTAGMSIVFVLLALSGVAALSLRRRSVH

SEQ ID NO: 12 - protein, 1795 aa, Bifidobacterium bifidum
  SOURCE 1..1795: /mol_type="protein" /note="gi|309252190|gb|ADO53938.1| sialidase [Bifidobacterium bif idum S17]" /organism="Bifidobacterium bifidum"
MTTIFRRATAKTLMRKLSGLLVAIAMLAVLPAGTISANAADEPPQEYLQLTLTRTDSNGTPAEVGDKLTYSLGYKNVSDTGFIVHPTASNLNNVATPQSASNPNPMCRWGNLAAGASAACTWSASKEFAYHVVTEDDVANGFTPTATVSATTQDGTNGVLQSVDITGETVPAVPATSTLRVAMQRTDTLGDNVKIGDRLTFNFTYTNKTAQKIYAYPSESNIERVDVVSFPRNSCRSGVEANQTASCGFAYHVITAEDVVARRYTPTATFRATSDRDGTQVLQDDMTFTTGTVTVAGPADDAASTPTERKDGEPLLLATNKQIGNTDYYRIPAIAQAPNGWILAAWDLRPKLAADAPNPNSIVQRISKDGGKSWETLAYVAQGRSATNKYGYSDPSYVVDEEAGKIFLFCVKSYDQGYFGSVLGVEDARNVLQAVVMESDDNGATWSEPRNITKDITKGHEDEWKSRFASSGHGIQLKYGQYKGRLIQQYAVRTTSNTNIAVSVYSDDHGKTWKAGNPVTEVNMDENKVVELSDGRVMLNSRPGAAGYRRVAISEDGGVNYGPIKSETQLPDPNNNAQITRAFPNAPEGSAKAKVLLYSAPRASNEGRANGVVRVSFDDGTTWSAGKLFKAGSMAYSVITALNDAAGGGYGLLYEGESITYTRASMEWLGYLTATASGTAAVKEGEGTLTAPVTVTNDGLTDYTNVTVTPTGLPSGWSAEAVNVGNLAAGQSATVNVPVTVPAAAVSGTVAKATMKITGKYAQSEDTLHSFAEGELAVTVTDPDPAAKRLKLTIERTDDNGDPVKVGDTLTYRITYENVGTQSFAVYPRESNLDGVTTPQSASNPAPVCRWSRLAPGATGACVSGNGKQLAYHTVTEADATAGSFTPSATIDATADASGETVLESVSITGDPVTVSQPVELPADIAAWKTRNEALADWQTLSEKLAKTDRINWLFTGDSITHGVQFTRGYRTYSELFANHLDTASVRGVSRANDVVMNTGISSADASWPLKDGAFEKWVSDKHPDVVFLTFGMNDGRTGQAFTVDQYTANLSTLIDKIRDLGAIPVLQTQNYTTNTTFNANLDTYFDAERRLALDKNVLLVDFNKQWLELGGGNRESGTYMGAGNDIHPGENGHIEWAKFTLGALNMIANDDPLARWSSSDTTLDKPTVTVDADGNGLKGSDGLEPAPAAAKSVGKFLSGAQYVDLGGDVVSAVAGKRESNVTIRFRASATGQPQTLFSLGDSDSATRATVRLSATGLVQFLNSGNTGDFYTVGTNDLADGAWHTVSVNFVANGFTIYVDGAAMRAISGGAGTQLNVPGAITVNTATAGAIRGADSAGGAQQLTGIVDYVAAWSRTLTDAEAKRISAETSAVAVTKVDAAVNALQPIISDTGARKNIVFVGGETIEGGYTDHLIAKNIVQLLDERVRWEYVTGLSATDRERQRAKFFVAAGQGGLTAKQMDEDYAAMVGEYSPDILFLAPDLYDADGNLAESAAAAFAGHIRSVAAKAKEAGAKVVLVTPVTVRGGEDEYAGAMRTVAKEDDLPLIDAQAWIGKVVAADASVKTAWFNKAGQLNYAGHLGYARFMMRSLDLYPSNVSGSRIASLPYDTANVTLVGASENGGELPVGRVEGTDRAHIDTMQIGAAASLVVVDSYAVYEIGEDGGRTLVADGLKPADVLADGIDVTVNDTAAHRYEVVGSANVPEGADAVTVTYTATLAAVEEPEPGPDPDPTPDPSEKPDGDGTGDGTGAGTGDVQKPTPDAVAKTGADVFGLLTAVAALLAAGGVTLSLRRRANR

SEQ ID NO: 13 - protein, 824 aa, Bifidobacterium longum subsp. infantis
  SOURCE 1..824: /mol_type="protein" /note="gi|213523006|gb|ACJ51753.1| glycosyl hydrolase, BNR repeat -containing protein [Bifidobacterium longum subsp. infantis ATCC 15697]" /organism="Bifidobacterium longum subsp. infantis"
MAASNPISWSQRTFPSPEGTIACRFRAHADGRIFDAVNGSANDAPLLICAIEHDALRVRATTPRQHVDFDIEDTTGIADGAMHTFALTFGEFGTRVYLDGSQCFSGTANLCPTTLTGTEGSGQGAIRLAGPSIDVTDMRLHAIPLTSESIAALTPRPAPDIDFAAAQLAPRDVRRVRTLRSGTIFMHFRVRGPRQYGTLLAAGERGEERLAVSIDDNGITMTAADGLYEPSTYHARGAWDDGRWHDLSIRSARGAIDMYVDGWHELHQAGQVFFGDWPQLDEVAIGQNTEGVRLMGEVRNGGVFTTPLTDGAIRRLSDAPALTTTALFDKGYHGSVSYRIPSIIRTPHGVVVAGADQRTAIANDAPNHINFVMRRSLDGGRTWLDMQTVIANPGEGVDGACTIDSCLVCDERNGRLTVLIDRFAGGVGLPNNTPGTGVDRHGRPCLYDRAGTRYVLADDGTVLDGGGERTGYRVDAHGNVTHEGRASGNIYLKEGADPDESLLIERTSFIIELHSDDDGETWSTPRNINHMIKEDWMHFLGVSPGNGIQLQASEHRGRLLVPFYCTGASLKHYSGGALISDDGGDTWRRGSMINDGRIVNGTAVDPKNIRDDDATTHESVFVERADGTVVCFFRNQNHAGRIGVALSHDGGETWDDLYFDKDVPDIFCQPNAVACAPRSDTMVFANASQMLPYRGNGVLRLSLDGARTWAAHRCINPYHYGYQCMTMLPDGELGLLWERETAGLYFTTLPLSVFGAAETHSADPEPKPEPKPEPEKPAGPKVDVPTEKPGLSKTGASTAGMSIVFVLLALSGVAALSLRRRSVH

SEQ ID NO: 14 - protein, 393 aa, Bifidobacterium longum subsp. infantis
  SOURCE 1..393: /mol_type="protein" /note="gi|213524659|gb|ACJ53406.1| Exo-alpha-sialidase [Bifidobac terium longum subsp. infantis ATCC 15697]" /organism="Bifidobacterium longum subsp. infantis"
MTENGMMNTNNTVCGANHDGAMSLAAPGDYGVACYRIPALAEAPNGWILAAFDARPHNCQDAPQANSIVQRISKDGGRSFEPQHVVAAGHDGVDKYGYSDPSYVVDRQTGEVFLFFVKSYDAGFGTSQAGVDPSAREVLQAAVTSSIDNGVTWSEPRIITADITNSESWISRFASSGAGIQLTYGEHAGRLIQQYTIKELDGRYRAVSVFSDDHGATWHAGTPVGDHMDENKVVELSDGRVMLNSRSSDGNGCRYVAISRDGGATYGPVIRETQLPDPENNAQIARAFPDAPEGSAQAKVLLYSSSSPSDRIDGLVRVSIDDGKTWSAGRRFTTGPMAYSVIAALSHKAGGGYGLLYEGDNNNIMYTRISLDWLNGQLNVDGIGGFPLSGEGG

SEQ ID NO: 15 - protein, 642 aa, Trypanosoma cruzi
  SOURCE 1..642: /mol_type="protein" /note="gi|432485|gb|AAA66352.1| trans-sialidase [Trypanosoma cruz i]" /organism="Trypanosoma cruzi"
MLAPGSSRVELFKRQSSKVPFEKDGKVTERVVHSFRLPALVNVDGVMVAIADARYETSNDNSLIDTVAKYSVDDGETWETQIAIKNSRASSVSRVVDPTVIVKGNKLYVLVGSYNSSRSYWTSHGDARDWDILLAVGEVTKSTAGGKITASIKWGSPVSLKEFFPAEMEGMHTNQFLGGAGVAIVASNGNLVYPVQVTNKKKQVFSKIFYSEDEGKTWKFGKGRSAFGCSEPVALEWEGKLIINTRVDYRRRLVYESSDMGNSWLEAVGTLSRVWGPSPKSNQPGSQSSFTAVTIEGMRVMLFTHPLNFKGRWLRDRLNLWLTDNQRIYNVGQVSIGDENSAYSSVLYKDDKLYCLHEINSNEVYSLVFARLVGELRIIKSVLQSWKNWDSHLSSICTPADPAASSSERGCGPAVTTVGLVGFLSHSATKTEWEDAYRCVNASTANAERVPNGLKFAGVGGGALWPVSQQGQNQRYRFANHAFTVVASVTIHEVPSVASPLLGASLDSSGGKKLLGLSYDERHQWQPIYGSTPVTPTGSWEMGKRYHVVLTMANKIGSEYIDGEPLEGSGQTVVPDERTPDISHFYVGGYKRSDMPTISHVTVNNVLLYNRQLNAEEIRTLFLSQDLIGTEAHMDSSSDTSA

SEQ ID NO: 16 - protein, 964 aa, Trypanosoma cruzi
  SOURCE 1..964: /mol_type="protein" /note="trans-sialidase enzyme of T. Cruzi, Uniprot accession no Q 26963-1" /organism="Trypanosoma cruzi"
MGKTVVGASRMFWLMFFVPLLLALCPSEPAHALAPGSSRVELFKRQSSKVPFEKGGKVTERVVHSFRLPALVNVDGVMVAIADARYETSNDNSLIDTVAKYSVDDGETWETQIAIKNSRASSVSRVVDPTVIVKGNKLYVLVGSYNSSRSYWTSHGDARDWDILLAVGEVTKSTAGGKITASIKWGSPVSLKEFFPAEMEGMHTNQFLGGAGVAIVASNGNLVYPVQVTNKKKQVFSKIFYSEDDGKTWKFGEGRSAFGCSEAVALEWEGKLIINTRVDYRRRLVYESSDMGNTWLEAVGTLSRVWGPSPKSNQPGSQSSFTAVTIEGMRVMLFTHPLNFKGRWLRDRLNLWLTDNQRIYNVGQVSIGDENSAHSSVLYKDDKLYCLHEINSNEVYSLVFARLVGELRIIKSVLQSWKNWDSHLSSICTPADPAASSSERGCGPAVTTVGLVGFLSHSATKTEWEDAYRCVNASTANAERVPNGLKFAGVGGGALWPVSQQGQNQRYHFANHAFTLVASVTIHEVPSVASPLLGASLDSSGGKKLLGLSYDEKHQWQPIYGSTPVTPTGSWETGKRYHVVLTMANKIGSVYIDGEPLEGSGQTVVPDGRTPDISHFYVGGYRRSDMPTISHVTVNNVLLYNRQLNAEEIRTLFLSQDLIGTEAHMDSSSDSNAHSTPSTPGDSSAHSTPSTPADNGAHSTPSTPADNGAHSTPSTPGDNGAHSTPLTPADNGAHSTPPTPADSSAHSTPSTPADNGAHSTPSTPADNGAHSTPLTPADNGAHSTPPTPADSSAHSTPSTPADNGAHSTPSTPADNGAHSTPPTPADSSAHSTPSTPGDNGAHSTPLTPADNGAHSTPLTPADSSAHSTPSTPGDNGAHSTPSAPADNGAHSTPPTPASNGAHSTPSAPGDNGAHSTPSTPADNDANGMVLFFPDGAAFSAFSGGGLLSCASALLLHVFVMAVLF

SEQ ID NO: 17 - protein, 1112 aa, Bifidobacterium bifidum
  SOURCE 1..1112: /mol_type="protein" /note="gi|167369738|gb|ABZ78855.1|lacto-N-biosidase[Bifidobacteri umbifidumJCM1254]" /organism="Bifidobacterium bifidum"
MEKSSNRRFGVRTVAAIVAGLMVGGMCTAMTASAADDSAAGYSATAPVNLTRPATVPSMDGWTDGTGAWTLGEGTRVVSSDALAARAQSLASELTKFTDVDIKAATGSATGKDISLTLDASKKAELGDEGFKLNIGSKGLEVIGATDIGVFYGTRSVSQMLRQGQLTLPAGTVATKPKYKERGATLCACQINISTDWIDRFLSDMADLRLNYVLLEMKLKPEEDNTKKAATWSYYTRDDVKKFVKKANNYGIDVIPEINSPGHMNVWLENYPEYQLADNSGRKDPNKLDISNPEAVKFYKTLIDEYDGVFTTKYWHMGADEYMIGTSFDNYSKLKTFAEKQYGAGATPNDAFTGFINDIDKYVKAKGKQLRIWNDGIVNTKNVSLNKDIVIEYWYGAGRKPQELVQDGYTLMNATQALYWSRSAQVYKVNAARLYNNNWNVGTFDGGRQIDKNYDKLTGAKVSIWPDSSYFQTENEVEKEIFDGMRFISQMTWSDSRPWATWNDMKADIDKIGYPLDIREYDYTPVDAGIYDIPQLKSISKGPWELITTPDGYYQMKDTVSGKCLALFTGSKHLDVVTQVGARPELRNCADVSVGQDQRNTANERNTQKWQIRADKDGKYTISPALTQQRLAIATGNEQNIDLETHRPAAGTVAQFPADLVSDNALFTLTGHMGMSATVDSKTVNPASPSKITVKVRAASNANTGDVTVTPVVPEGWEIKPGSVSLKSIPAGKAAIAYFNVVNTTGTGDATVQFKLTNTKTGEELGTTSVALTGSLTKDVEASDYAASSQETTGEHAPVGNAFDKNANTFWHSKYSNPSANLPHWLAFKASPGEGNKIAAITHLYRQDKLNGPAKNVAVYVVAASDANSVADVTNWGEPVATAEFPYTKELQTIALPNTIPSGDVYVKFQINDAWGLTETSAGVTWAAVAELAATAKATPVELTEPEQPKDNPEVTETPEATGVTVSGDGVANGALSLKKGTTAQLTAKVAPDDADQAVTWASSDDKVVTVDKTGKVTAVAKGVAKVTATTANGKSASVTVTVTEDSEVPGPTGPTEPTKPGTEKPTTKPTTKPNDGKLSATGADTAVLATIAALFALAGGAVVAVRRRSVR

SEQ ID NO: 18 - protein, 639 aa, Streptomyces sp.
  SOURCE 1..639: /mol_type="protein" /note="gi|4096812|gb|AAD10478.1|lacto-N-biosidaseprecursor[Strept omycessp.]" /organism="Streptomyces sp."
MDMRMARRRTIGAVVTALAAALLPWQSATAEGGSAAAAPPEVLPTLREWQGGQGEFTLTDRAGIVLDGVRDSRTAADARRFAGELNGKASVSQGRAARPGDIVLRQDPAQKGLLGAEGYRLTVGTRITVTAATSTGVFYGTRTVLQLLNDDGRAARGSATDVPAYRERGVGVCACYINISTQWFERLMKDMASQKLNQLWIEAKVKSDTDPASAFWGYYTKPQVRTLVAMARKYHIELVPEINSPGHMDTYLENHPELQLKDRDGVASPPRLDISRPEALAYYTSMVDEALKVWDSRYWHMGADEYMIGSSYPDYPQLQAAARAKFGASATPDDLFTDFINQVNAHVKADGRSLRIWNDGLAGKNAVVPLDRDITVEHWLSGGSIQQPSSLLAEGRPVMNSAYSLYLVRGGFTMQTQKLYESDWTPLRFEGQTLTQGAANLTGAKISLWPDSAAAETENEVETKVFMPLRFVAQATWGGPKPSPTYAGFEALARKIGHAPGWENTDRTPLADGTYRLTTGAKALAPTADAGVSLVKNSAASWALTATADGYYTVRSTESGQCLDAVRGKKYLGAPLEVGAELSLANCSTTARTQRWQLDTGAGALTLRNAISQLHLTERASDGAAVQTTGATRLTARAA

SEQ ID NO: 19 - protein, 699 aa, Bacillus circulans
  SOURCE 1..699: /mol_type="protein" /note="gi|142688|gb|AAA81528.1|chitinaseA1[Bacilluscirculans]" /organism="Bacillus circulans"
MINLNKHTAFKKTAKFFLGLSLLLSVIVPSFALQPATAEAADSYKIVGYYPSWAAYGRNYNVADIDPTKVTHINYAFADICWNGIHGNPDPSGPNPVTWTCQNEKSQTINVPNGTIVLGDPWIDTGKTFAGDTWDQPIAGNINQLNKLKQTNPNLKTIISVGGWTWSNRFSDVAATAATREVFANSAVDFLRKYNFDGVDLDWEYPVSGGLDGNSKRPEDKQNYTLLLSKIREKLDAAGAVDGKKYLLTIASGASATYAANTELAKIAAIVDWINIMTYDFNGAWQKISAHNAPLNYDPAASAAGVPDANTFNVAAGAQGHLDAGVPAAKLVLGVPFYGRGWDGCAQAGNGQYQTCTGGSSVGTWEAGSFDFYDLEANYINKNGYTRYWNDTAKVPYLYNASNKRFISYDDAESVGYKTAYIKSKGLGGAMFWELSGDRNKTLQNKLKADLPTGGTVPPVDTTAPSVPGNARSTGVTANSVTLAWNASTDNVGVTGYNVYNGANLATSVTGTTATISGLTAGTSYTFTIKAKDAAGNLSAASNAVTVSTTAQPGGDTQAPTAPTNLASTAQTTSSITLSWTASTDNVGVTGYDVYNGTALATTVTGTTATISGLAADTSYTFTVKAKDAAGNVSAASNAVSVKTAAETTNPGVSAWQVNTAYTAGQLVTYNGKTYKCLQPHTSLAGWEPSNVPALWQLQ

SEQ ID NO: 20 - protein, 702 aa, Trypanosoma congolense
  SOURCE 1..702: /mol_type="protein" /note="gi|343957998|emb|CCD30509.1| trans-sialidase [Trypanosoma congolense]" /organism="Trypanosoma congolense"
QCCDHMHATAAVGTTHQALLWGSKWALRNKTTPKDGEVWWSNPQPGWKEVYDDEWEEWFMEQKGPTGVNGVRTEWYRRMKDGYILVGGPKLNSPDMNSTGTTMRTVHSYRIPSIVEVGGVLMCVGDARYITSTDYFFTDTVAAYSTDGGRTWKREVIIPNGRVDAHYSRVVDPTVVAKGNNIYVLVGRYNVTRGYWHNKNNRAGVADWEPFVYKGTVNVGTKDNATDVSISWERTALKSLYNFPVSGSPGTQFLGGAGGGVVTSNGTIVLPVQARNKANRVVSMILYSADDGKSWHFGKGEAGVGTSEAALTEWDGKLLISARSDGGQGYRMIFESSDLGATWKEMLNSISRVIGNSPGRSGPGSSSGFITVTVEGVPVMLLTHPKNLKGSYYRDRLQMWMTDGNRMWHVGQVSEGDDNSAYSSLLYTPDGVLYCLHEQNIDEVYSLHLVRLVDELKSIKSTALVWKAQDELLLGNCLPGDKYDPGCDGIPTAGLAGLLVGPLTEKTWPDAYRCVNAATSGAVSTAEGVRLDVGGGGHVVWPVSEQGQDQRYYFTNSEFTLAVTVRFDEMPQGELPLLGFVNREGKVKKILKVSLSGVEWLLAYGNEYNSTAAEPLDVNESHQVVLALHDGIVSLHVDGGNTTATVSVRVASPAELLNIHHLFVGTPVDGGAKEHANITVSNVLVYNRPLRGVELLGLFANR

SEQ ID NO: 21 - protein, 702 aa, Trypanosoma congolense
  SOURCE 1..702: /mol_type="protein" /note="gi|343958004|emb|CCD30512.1| trans-sialidase [Trypanosoma congolense]" /organism="Trypanosoma congolense"
QCCDHMHATAAVGTTHQALLWGSKWALRNKTTPKDGEVWWSNPQPGWKEVYDDEWEEWFMEQEGPTGVNGVRGEWYRRMTDGYILVGGPKLNSPDMNSTGTTMRTVHSYRIPSIVEVGGVLMCVGDARYITSTDYFFTDTVAAYSTDGGRTWKREVIIPNGRVDAHYSRVVDPTVVAKGNNIYVLVGRYNVTRGYWHNKNNRAGVADWEPFVYKGTVNVGTKDNATDVSISWERTALKSLYNFPVSGSPGTQFLGGAGGGVVTSNGTIVLPVQARNKANRVVSMILYSADDGKSWHFGKGEAGVGTSEAALTEWDGKLLISARSDGGQGYRMIFESSDLGATWKEMLNSISRVIGNSPGRSGPGSSSGFITVTVEGVPVMLLTHPKNFKGSYYRDRLQMWMTDGNRMWHVGQVSEGDDNSAYSSLLYTPDGVLYCLHEQNIDEVYSLHLVRLVDELKSIKSTALVWKAQDELLLGNCLPGDKYDPGCDGIPTAGLAGLLVGPLTEKTWPDAYRCVNAATSGAVSTAEGVRLDVGGGGHVVWPVSEQGQDQRYYFTNSEFTLAVTVRFDEMPHGELPLLGFVNRKDQVKKILKVSLSGVEWLLAYGNEYNSTAAEPLNVNESHQVVLTLHDGIVSLHVDGGNMTATVSVRVASPAELLNIHHLFVGTPVDGGAKEHANITVSNVLVYNRPLRGVELLGLFANR